European Patent Application EP 4 151 648 A1, published March 22, 2023. Title: SYSTEME D'EXPRESSION BACULOVIRUS. Applicant: CENTRE NATIONAL DE LA RECHERCHE SCIENTIFIQUE (CNRS). The sequence listing filed with the application follows.

SEQUENCE LISTING (3 sequences)

SEQ ID NO: 1 - DNA, 75 bp, synthetic construct
  misc_feature 1..75: note = P10 sauvage
  source 1..75: mol_type = other DNA
ataagaattattatcaaatcatttgtatattaattaaaatactatactgtaaattacattttatttacaatcatg

SEQ ID NO: 2 - DNA, 71 bp, synthetic construct
  misc_feature 1..71: note = P10S1A
  source 1..71: mol_type = other DNA
ataagtattttaatcttttcgtttgtataaattaatttatactatactgtataaaaaaacctataaatatg

SEQ ID NO: 3 - DNA, 71 bp, synthetic construct
  misc_feature 1..71: note = P10S1B
  source 1..71: mol_type = other DNA
ataagtattttaatcttttcgtttgtaccactgcagtggtactatactgtataaaaaaacctataaatatg